European Patent Application EP 4 368 717 A1, published May 15, 2024. Title: MARC1 유전자를 표적으로 하는 RNAi 제제 및 이의 용도. Applicant: 올릭스(주). Application KP. The sequence listing filed with the application follows.

SEQUENCE LISTING (600 sequences)

SEQ ID NO: 1 - RNA, 16 nt, synthetic construct
  source 1..16: mol_type = other RNA
gctctggatctaccct

SEQ ID NO: 2 - RNA, 19 nt, synthetic construct
  source 1..19: mol_type = other RNA
agggtagatccagagctgc

SEQ ID NO: 3 - RNA, 16 nt, synthetic construct
  source 1..16: mol_type = other RNA
cagctctggatctacc

SEQ ID NO: 4 - RNA, 19 nt, synthetic construct
  source 1..19: mol_type = other RNA
ggtagatccagagctgcgc

SEQ ID NO: 5 - RNA, 16 nt, synthetic construct
  source 1..16: mol_type = other RNA
gcagctctggatctac

SEQ ID NO: 6 - RNA, 19 nt, synthetic construct
  source 1..19: mol_type = other RNA
gtagatccagagctgcgcc

SEQ ID NO: 7 - RNA, 16 nt, synthetic construct
  source 1..16: mol_type = other RNA
gccatggggctgcgca

SEQ ID NO: 8 - RNA, 19 nt, synthetic construct
  source 1..19: mol_type = other RNA
tgcgcagccccatggccgt

SEQ ID NO: 9 - RNA, 16 nt, synthetic construct
  source 1..16: mol_type = other RNA
ggccatggggctgcgc

SEQ ID NO: 10 - RNA, 19 nt, synthetic construct
  source 1..19: mol_type = other RNA
gcgcagccccatggccgtg

SEQ ID NO: 11 - RNA, 16 nt, synthetic construct
  source 1..16: mol_type = other RNA
cggccatggggctgcg

SEQ ID NO: 12 - RNA, 19 nt, synthetic construct
  source 1..19: mol_type = other RNA
cgcagccccatggccgtgc

SEQ ID NO: 13 - RNA, 16 nt, synthetic construct
  source 1..16: mol_type = other RNA
acggccatggggctgc

SEQ ID NO: 14 - RNA, 19 nt, synthetic construct
  source 1..19: mol_type = other RNA
gcagccccatggccgtgca

SEQ ID NO: 15 - RNA, 16 nt, synthetic construct
  source 1..16: mol_type = other RNA
cacggccatggggctg

SEQ ID NO: 16 - RNA, 19 nt, synthetic construct
  source 1..19: mol_type = other RNA
cagccccatggccgtgcac

SEQ ID NO: 17 - RNA, 16 nt, synthetic construct
  source 1..16: mol_type = other RNA
ggacaggttttggctt

SEQ ID NO: 18 - RNA, 19 nt, synthetic construct
  source 1..19: mol_type = other RNA
aagccaaaacctgtcccgc

SEQ ID NO: 19 - RNA, 16 nt, synthetic construct
  source 1..16: mol_type = other RNA
gggacaggttttggct

SEQ ID NO: 20 - RNA, 19 nt, synthetic construct
  source 1..19: mol_type = other RNA
agccaaaacctgtcccgca

SEQ ID NO: 21 - RNA, 16 nt, synthetic construct
  source 1..16: mol_type = other RNA
cgggacaggttttggc

SEQ ID NO: 22 - RNA, 19 nt, synthetic construct
  source 1..19: mol_type = other RNA
gccaaaacctgtcccgcag

SEQ ID NO: 23 - RNA, 16 nt, synthetic construct
  source 1..16: mol_type = other RNA
agcctacacaaaggac

SEQ ID NO: 24 - RNA, 19 nt, synthetic construct
  source 1..19: mol_type = other RNA
gtcctttgtgtaggctgca

SEQ ID NO: 25 - RNA, 16 nt, synthetic construct
  source 1..16: mol_type = other RNA
ggtgcacttcgagcct

SEQ ID NO: 26 - RNA, 19 nt, synthetic construct
  source 1..19: mol_type = other RNA
aggctcgaagtgcaccagg

SEQ ID NO: 27 - RNA, 16 nt, synthetic construct
  source 1..16: mol_type = other RNA
ctggtgcacttcgagc

SEQ ID NO: 28 - RNA, 19 nt, synthetic construct
  source 1..19: mol_type = other RNA
gctcgaagtgcaccaggcg

SEQ ID NO: 29 - RNA, 16 nt, synthetic construct
  source 1..16: mol_type = other RNA
cctggtgcacttcgag

SEQ ID NO: 30 - RNA, 19 nt, synthetic construct
  source 1..19: mol_type = other RNA
ctcgaagtgcaccaggcgg

SEQ ID NO: 31 - RNA, 16 nt, synthetic construct
  source 1..16: mol_type = other RNA
gcctggtgcacttcga

SEQ ID NO: 32 - RNA, 19 nt, synthetic construct
  source 1..19: mol_type = other RNA
tcgaagtgcaccaggcggt

SEQ ID NO: 33 - RNA, 16 nt, synthetic construct
  source 1..16: mol_type = other RNA
cgcctggtgcacttcg

SEQ ID NO: 34 - RNA, 19 nt, synthetic construct
  source 1..19: mol_type = other RNA
cgaagtgcaccaggcggta

SEQ ID NO: 35 - RNA, 16 nt, synthetic construct
  source 1..16: mol_type = other RNA
ccgcctggtgcacttc

SEQ ID NO: 36 - RNA, 19 nt, synthetic construct
  source 1..19: mol_type = other RNA
gaagtgcaccaggcggtag

SEQ ID NO: 37 - RNA, 16 nt, synthetic construct
  source 1..16: mol_type = other RNA
accgcctggtgcactt

SEQ ID NO: 38 - RNA, 19 nt, synthetic construct
  source 1..19: mol_type = other RNA
aagtgcaccaggcggtagg

SEQ ID NO: 39 - RNA, 16 nt, synthetic construct
  source 1..16: mol_type = other RNA
taccgcctggtgcact

SEQ ID NO: 40 - RNA, 19 nt, synthetic construct
  source 1..19: mol_type = other RNA
agtgcaccaggcggtaggg

SEQ ID NO: 41 - RNA, 16 nt, synthetic construct
  source 1..16: mol_type = other RNA
ctaccgcctggtgcac

SEQ ID NO: 42 - RNA, 19 nt, synthetic construct
  source 1..19: mol_type = other RNA
gtgcaccaggcggtagggc

SEQ ID NO: 43 - RNA, 16 nt, synthetic construct
  source 1..16: mol_type = other RNA
gacgtggaactgaaaa

SEQ ID NO: 44 - RNA, 19 nt, synthetic construct
  source 1..19: mol_type = other RNA
ttttcagttccacgtcacc

SEQ ID NO: 45 - RNA, 16 nt, synthetic construct
  source 1..16: mol_type = other RNA
tgacgtggaactgaaa

SEQ ID NO: 46 - RNA, 19 nt, synthetic construct
  source 1..19: mol_type = other RNA
tttcagttccacgtcacca

SEQ ID NO: 47 - RNA, 16 nt, synthetic construct
  source 1..16: mol_type = other RNA
ggaaacactgaagagt

SEQ ID NO: 48 - RNA, 19 nt, synthetic construct
  source 1..19: mol_type = other RNA
actcttcagtgtttccagc

SEQ ID NO: 49 - RNA, 16 nt, synthetic construct
  source 1..16: mol_type = other RNA
tggaaacactgaagag

SEQ ID NO: 50 - RNA, 19 nt, synthetic construct
  source 1..19: mol_type = other RNA
ctcttcagtgtttccagcg

SEQ ID NO: 51 - RNA, 16 nt, synthetic construct
  source 1..16: mol_type = other RNA
ctggaaacactgaaga

SEQ ID NO: 52 - RNA, 19 nt, synthetic construct
  source 1..19: mol_type = other RNA
tcttcagtgtttccagcgg

SEQ ID NO: 53 - RNA, 16 nt, synthetic construct
  source 1..16: mol_type = other RNA
gctggaaacactgaag

SEQ ID NO: 54 - RNA, 19 nt, synthetic construct
  source 1..19: mol_type = other RNA
cttcagtgtttccagcggt

SEQ ID NO: 55 - RNA, 16 nt, synthetic construct
  source 1..16: mol_type = other RNA
cgctggaaacactgaa

SEQ ID NO: 56 - RNA, 19 nt, synthetic construct
  source 1..19: mol_type = other RNA
ttcagtgtttccagcggtt

SEQ ID NO: 57 - RNA, 16 nt, synthetic construct
  source 1..16: mol_type = other RNA
ccgctggaaacactga

SEQ ID NO: 58 - RNA, 19 nt, synthetic construct
  source 1..19: mol_type = other RNA
tcagtgtttccagcggttc

SEQ ID NO: 59 - RNA, 16 nt, synthetic construct
  source 1..16: mol_type = other RNA
cgcagctctggatcta

SEQ ID NO: 60 - RNA, 19 nt, synthetic construct
  source 1..19: mol_type = other RNA
tagatccagagctgcgcca

SEQ ID NO: 61 - RNA, 16 nt, synthetic construct
  source 1..16: mol_type = other RNA
gcgcagctctggatct

SEQ ID NO: 62 - RNA, 19 nt, synthetic construct
  source 1..19: mol_type = other RNA
agatccagagctgcgccac

SEQ ID NO: 63 - RNA, 16 nt, synthetic construct
  source 1..16: mol_type = other RNA
ggcgcagctctggatc

SEQ ID NO: 64 - RNA, 19 nt, synthetic construct
  source 1..19: mol_type = other RNA
gatccagagctgcgccact

SEQ ID NO: 65 - RNA, 16 nt, synthetic construct
  source 1..16: mol_type = other RNA
gccggtgagcgaggcg

SEQ ID NO: 66 - RNA, 19 nt, synthetic construct
  source 1..19: mol_type = other RNA
cgcctcgctcaccggcacc

SEQ ID NO: 67 - RNA, 16 nt, synthetic construct
  source 1..16: mol_type = other RNA
cctggtcctgatttcc

SEQ ID NO: 68 - RNA, 19 nt, synthetic construct
  source 1..19: mol_type = other RNA
ggaaatcaggaccaggcga

SEQ ID NO: 69 - RNA, 16 nt, synthetic construct
  source 1..16: mol_type = other RNA
gcctggtcctgatttc

SEQ ID NO: 70 - protein, 19 aa, synthetic construct
GAAATCAGGACCAGGCGAG

SEQ ID NO: 71 - RNA, 16 nt, synthetic construct
  source 1..16: mol_type = other RNA
cgcctggtcctgattt

SEQ ID NO: 72 - RNA, 19 nt, synthetic construct
  source 1..19: mol_type = other RNA
aaatcaggaccaggcgagg

SEQ ID NO: 73 - RNA, 16 nt, synthetic construct
  source 1..16: mol_type = other RNA
tgactctcagtgcagc

SEQ ID NO: 74 - RNA, 19 nt, synthetic construct
  source 1..19: mol_type = other RNA
gctgcactgagagtcaggg

SEQ ID NO: 75 - RNA, 16 nt, synthetic construct
  source 1..16: mol_type = other RNA
ctgactctcagtgcag

SEQ ID NO: 76 - RNA, 19 nt, synthetic construct
  source 1..19: mol_type = other RNA
ctgcactgagagtcagggt

SEQ ID NO: 77 - RNA, 16 nt, synthetic construct
  source 1..16: mol_type = other RNA
cctgactctcagtgca

SEQ ID NO: 78 - RNA, 19 nt, synthetic construct
  source 1..19: mol_type = other RNA
tgcactgagagtcagggtg

SEQ ID NO: 79 - RNA, 16 nt, synthetic construct
  source 1..16: mol_type = other RNA
ccctgactctcagtgc

SEQ ID NO: 80 - RNA, 19 nt, synthetic construct
  source 1..19: mol_type = other RNA
gcactgagagtcagggtgt

SEQ ID NO: 81 - RNA, 16 nt, synthetic construct
  source 1..16: mol_type = other RNA
accctgactctcagtg

SEQ ID NO: 82 - RNA, 19 nt, synthetic construct
  source 1..19: mol_type = other RNA
cactgagagtcagggtgtc

SEQ ID NO: 83 - RNA, 16 nt, synthetic construct
  source 1..16: mol_type = other RNA
gcacggcctggagata

SEQ ID NO: 84 - RNA, 19 nt, synthetic construct
  source 1..19: mol_type = other RNA
tatctccaggccgtgcact

SEQ ID NO: 85 - RNA, 16 nt, synthetic construct
  source 1..16: mol_type = other RNA
gatcctttctgaggcg

SEQ ID NO: 86 - RNA, 19 nt, synthetic construct
  source 1..19: mol_type = other RNA
cgcctcagaaaggatcaag

SEQ ID NO: 87 - RNA, 16 nt, synthetic construct
  source 1..16: mol_type = other RNA
tgatcctttctgaggc

SEQ ID NO: 88 - RNA, 19 nt, synthetic construct
  source 1..19: mol_type = other RNA
gcctcagaaaggatcaaga

SEQ ID NO: 89 - RNA, 16 nt, synthetic construct
  source 1..16: mol_type = other RNA
tctcaactccaggcta

SEQ ID NO: 90 - RNA, 19 nt, synthetic construct
  source 1..19: mol_type = other RNA
tagcctggagttgagatcc

SEQ ID NO: 91 - RNA, 16 nt, synthetic construct
  source 1..16: mol_type = other RNA
atctcaactccaggct

SEQ ID NO: 92 - RNA, 19 nt, synthetic construct
  source 1..19: mol_type = other RNA
agcctggagttgagatccg

SEQ ID NO: 93 - RNA, 16 nt, synthetic construct
  source 1..16: mol_type = other RNA
ggatctcaactccagg

SEQ ID NO: 94 - RNA, 19 nt, synthetic construct
  source 1..19: mol_type = other RNA
cctggagttgagatccgcc

SEQ ID NO: 95 - RNA, 16 nt, synthetic construct
  source 1..16: mol_type = other RNA
cggatctcaactccag

SEQ ID NO: 96 - RNA, 19 nt, synthetic construct
  source 1..19: mol_type = other RNA
ctggagttgagatccgcca

SEQ ID NO: 97 - RNA, 16 nt, synthetic construct
  source 1..16: mol_type = other RNA
gcggatctcaactcca

SEQ ID NO: 98 - RNA, 19 nt, synthetic construct
  source 1..19: mol_type = other RNA
tggagttgagatccgccag

SEQ ID NO: 99 - RNA, 16 nt, synthetic construct
  source 1..16: mol_type = other RNA
agggtgatggcttgtt

SEQ ID NO: 100 - RNA, 19 nt, synthetic construct
  source 1..19: mol_type = other RNA
aacaagccatcaccctttt

SEQ ID NO: 101 - RNA, 16 nt, synthetic construct
  source 1..16: mol_type = other RNA
gagggaaacatggtta

SEQ ID NO: 102 - RNA, 21 nt, synthetic construct
  source 1..21: mol_type = other RNA
taaccatgtttccctcctggt

SEQ ID NO: 103 - RNA, 16 nt, synthetic construct
  source 1..16: mol_type = other RNA
ggagggaaacatggta

SEQ ID NO: 104 - RNA, 21 nt, synthetic construct
  source 1..21: mol_type = other RNA
taccatgtttccctcctggtt

SEQ ID NO: 105 - RNA, 16 nt, synthetic construct
  source 1..16: mol_type = other RNA
accaggagggaaacaa

SEQ ID NO: 106 - RNA, 21 nt, synthetic construct
  source 1..21: mol_type = other RNA
ttgtttccctcctggttgatc

SEQ ID NO: 107 - RNA, 16 nt, synthetic construct
  source 1..16: mol_type = other RNA
tcaaccaggagggaaa

SEQ ID NO: 108 - RNA, 21 nt, synthetic construct
  source 1..21: mol_type = other RNA
tttccctcctggttgatcaca

SEQ ID NO: 109 - RNA, 16 nt, synthetic construct
  source 1..16: mol_type = other RNA
ggcttgtgatcaacca

SEQ ID NO: 110 - RNA, 21 nt, synthetic construct
  source 1..21: mol_type = other RNA
tggttgatcacaagccaaaac

SEQ ID NO: 111 - RNA, 16 nt, synthetic construct
  source 1..16: mol_type = other RNA
gtcctgatttccctga

SEQ ID NO: 112 - RNA, 21 nt, synthetic construct
  source 1..21: mol_type = other RNA
tcagggaaatcaggaccaggc

SEQ ID NO: 113 - RNA, 16 nt, synthetic construct
  source 1..16: mol_type = other RNA
ctcgcctggtcctgaa

SEQ ID NO: 114 - RNA, 21 nt, synthetic construct
  source 1..21: mol_type = other RNA
ttcaggaccaggcgaggttcc

SEQ ID NO: 115 - RNA, 16 nt, synthetic construct
  source 1..16: mol_type = other RNA
cctcgcctggtcctga

SEQ ID NO: 116 - RNA, 21 nt, synthetic construct
  source 1..21: mol_type = other RNA
tcaggaccaggcgaggttcct

SEQ ID NO: 117 - RNA, 16 nt, synthetic construct
  source 1..16: mol_type = other RNA
gacaccctgactctca

SEQ ID NO: 118 - RNA, 21 nt, synthetic construct
  source 1..21: mol_type = other RNA
tgagagtcagggtgtcaccat

SEQ ID NO: 119 - RNA, 16 nt, synthetic construct
  source 1..16: mol_type = other RNA
tggtgacaccctgaca

SEQ ID NO: 120 - RNA, 21 nt, synthetic construct
  source 1..21: mol_type = other RNA
tgtcagggtgtcaccatcgca

SEQ ID NO: 121 - RNA, 16 nt, synthetic construct
  source 1..16: mol_type = other RNA
gcgatggtgacaccca

SEQ ID NO: 122 - RNA, 21 nt, synthetic construct
  source 1..21: mol_type = other RNA
tgggtgtcaccatcgcaggtc

SEQ ID NO: 123 - RNA, 16 nt, synthetic construct
  source 1..16: mol_type = other RNA
ccaccacaaatgcaga

SEQ ID NO: 124 - RNA, 21 nt, synthetic construct
  source 1..21: mol_type = other RNA
tctgcatttgtggtgggcgtt

SEQ ID NO: 125 - RNA, 16 nt, synthetic construct
  source 1..16: mol_type = other RNA
gcccaccacaaatgca

SEQ ID NO: 126 - RNA, 21 nt, synthetic construct
  source 1..21: mol_type = other RNA
tgcatttgtggtgggcgtttt

SEQ ID NO: 127 - protein, 16 aa, synthetic construct
AACGCCCACCACAAAA

SEQ ID NO: 128 - RNA, 21 nt, synthetic construct
  source 1..21: mol_type = other RNA
ttttgtggtgggcgttttgat

SEQ ID NO: 129 - RNA, 16 nt, synthetic construct
  source 1..16: mol_type = other RNA
tgcacaagtgcagaga

SEQ ID NO: 130 - RNA, 21 nt, synthetic construct
  source 1..21: mol_type = other RNA
tctctgcacttgtgcactgca

SEQ ID NO: 131 - RNA, 16 nt, synthetic construct
  source 1..16: mol_type = other RNA
gcttcctgaagtcaca

SEQ ID NO: 132 - RNA, 21 nt, synthetic construct
  source 1..21: mol_type = other RNA
tgtgacttcaggaagctggtt

SEQ ID NO: 133 - RNA, 16 nt, synthetic construct
  source 1..16: mol_type = other RNA
cagcttcctgaagtca

SEQ ID NO: 134 - RNA, 21 nt, synthetic construct
  source 1..21: mol_type = other RNA
tgacttcaggaagctggttat

SEQ ID NO: 135 - RNA, 16 nt, synthetic construct
  source 1..16: mol_type = other RNA
accagcttcctgaaga

SEQ ID NO: 136 - RNA, 21 nt, synthetic construct
  source 1..21: mol_type = other RNA
tcttcaggaagctggttatcc

SEQ ID NO: 137 - RNA, 16 nt, synthetic construct
  source 1..16: mol_type = other RNA
gcccagtggataacca

SEQ ID NO: 138 - RNA, 21 nt, synthetic construct
  source 1..21: mol_type = other RNA
tggttatccactgggcggtgg

SEQ ID NO: 139 - RNA, 16 nt, synthetic construct
  source 1..16: mol_type = other RNA
accgcccagtggataa

SEQ ID NO: 140 - RNA, 21 nt, synthetic construct
  source 1..21: mol_type = other RNA
ttatccactgggcggtggcct

SEQ ID NO: 141 - RNA, 16 nt, synthetic construct
  source 1..16: mol_type = other RNA
cacttcgagcctcaca

SEQ ID NO: 142 - RNA, 21 nt, synthetic construct
  source 1..21: mol_type = other RNA
tgtgaggctcgaagtgcacca

SEQ ID NO: 143 - RNA, 16 nt, synthetic construct
  source 1..16: mol_type = other RNA
tgcacttcgagcctca

SEQ ID NO: 144 - RNA, 21 nt, synthetic construct
  source 1..21: mol_type = other RNA
tgaggctcgaagtgcaccagg

SEQ ID NO: 145 - RNA, 16 nt, synthetic construct
  source 1..16: mol_type = other RNA
gacaccagcccattca

SEQ ID NO: 146 - RNA, 21 nt, synthetic construct
  source 1..21: mol_type = other RNA
tgaatgggctggtgtctgagt

SEQ ID NO: 147 - RNA, 16 nt, synthetic construct
  source 1..16: mol_type = other RNA
cagacaccagcccata

SEQ ID NO: 148 - RNA, 21 nt, synthetic construct
  source 1..21: mol_type = other RNA
tatgggctggtgtctgagtaa

SEQ ID NO: 149 - RNA, 16 nt, synthetic construct
  source 1..16: mol_type = other RNA
ccagattgcttactca

SEQ ID NO: 150 - RNA, 21 nt, synthetic construct
  source 1..21: mol_type = other RNA
tgagtaagcaatctggtcctt

SEQ ID NO: 151 - RNA, 16 nt, synthetic construct
  source 1..16: mol_type = other RNA
gaccagattgcttaca

SEQ ID NO: 152 - RNA, 21 nt, synthetic construct
  source 1..21: mol_type = other RNA
tgtaagcaatctggtccttgg

SEQ ID NO: 153 - RNA, 16 nt, synthetic construct
  source 1..16: mol_type = other RNA
aggaccagattgctta

SEQ ID NO: 154 - RNA, 21 nt, synthetic construct
  source 1..21: mol_type = other RNA
taagcaatctggtccttgggt

SEQ ID NO: 155 - RNA, 16 nt, synthetic construct
  source 1..16: mol_type = other RNA
acccaaggaccagata

SEQ ID NO: 156 - RNA, 21 nt, synthetic construct
  source 1..21: mol_type = other RNA
tatctggtccttgggtcggaa

SEQ ID NO: 157 - RNA, 16 nt, synthetic construct
  source 1..16: mol_type = other RNA
gacccaaggaccagaa

SEQ ID NO: 158 - RNA, 21 nt, synthetic construct
  source 1..21: mol_type = other RNA
ttctggtccttgggtcggaac

SEQ ID NO: 159 - RNA, 16 nt, synthetic construct
  source 1..16: mol_type = other RNA
gcgatgtctatgcaga

SEQ ID NO: 160 - RNA, 21 nt, synthetic construct
  source 1..21: mol_type = other RNA
tctgcatagacatcgcatcct

SEQ ID NO: 161 - RNA, 16 nt, synthetic construct
  source 1..16: mol_type = other RNA
aggatgcgatgtctaa

SEQ ID NO: 162 - RNA, 21 nt, synthetic construct
  source 1..21: mol_type = other RNA
ttagacatcgcatcctgaaat

SEQ ID NO: 163 - RNA, 16 nt, synthetic construct
  source 1..16: mol_type = other RNA
caggatgcgatgtcta

SEQ ID NO: 164 - RNA, 21 nt, synthetic construct
  source 1..21: mol_type = other RNA
tagacatcgcatcctgaaatt

SEQ ID NO: 165 - RNA, 16 nt, synthetic construct
  source 1..16: mol_type = other RNA
cccaatattgtaatta

SEQ ID NO: 166 - RNA, 21 nt, synthetic construct
  source 1..21: mol_type = other RNA
taattacaatattgggcctga

SEQ ID NO: 167 - RNA, 16 nt, synthetic construct
  source 1..16: mol_type = other RNA
gcccaatattgtaata

SEQ ID NO: 168 - RNA, 21 nt, synthetic construct
  source 1..21: mol_type = other RNA
tattacaatattgggcctgaa

SEQ ID NO: 169 - RNA, 16 nt, synthetic construct
  source 1..16: mol_type = other RNA
ggcccaatattgtaaa

SEQ ID NO: 170 - RNA, 21 nt, synthetic construct
  source 1..21: mol_type = other RNA
tttacaatattgggcctgaag

SEQ ID NO: 171 - RNA, 16 nt, synthetic construct
  source 1..16: mol_type = other RNA
acttcaggcccaataa

SEQ ID NO: 172 - RNA, 21 nt, synthetic construct
  source 1..21: mol_type = other RNA
ttattgggcctgaagttggtt

SEQ ID NO: 173 - RNA, 16 nt, synthetic construct
  source 1..16: mol_type = other RNA
aacttcaggcccaata

SEQ ID NO: 174 - RNA, 21 nt, synthetic construct
  source 1..21: mol_type = other RNA
tattgggcctgaagttggttg

SEQ ID NO: 175 - RNA, 16 nt, synthetic construct
  source 1..16: mol_type = other RNA
caacttcaggcccaaa

SEQ ID NO: 176 - RNA, 21 nt, synthetic construct
  source 1..21: mol_type = other RNA
tttgggcctgaagttggttgc

SEQ ID NO: 177 - RNA, 16 nt, synthetic construct
  source 1..16: mol_type = other RNA
ccaacttcaggcccaa

SEQ ID NO: 178 - RNA, 21 nt, synthetic construct
  source 1..21: mol_type = other RNA
ttgggcctgaagttggttgct

SEQ ID NO: 179 - RNA, 16 nt, synthetic construct
  source 1..16: mol_type = other RNA
agagaagaaagttaaa

SEQ ID NO: 180 - RNA, 21 nt, synthetic construct
  source 1..21: mol_type = other RNA
tttaactttcttctctagcct

SEQ ID NO: 181 - RNA, 16 nt, synthetic construct
  source 1..16: mol_type = other RNA
tagagaagaaagttaa

SEQ ID NO: 182 - RNA, 21 nt, synthetic construct
  source 1..21: mol_type = other RNA
ttaactttcttctctagcctg

SEQ ID NO: 183 - RNA, 16 nt, synthetic construct
  source 1..16: mol_type = other RNA
ctagagaagaaagtta

SEQ ID NO: 184 - RNA, 21 nt, synthetic construct
  source 1..21: mol_type = other RNA
taactttcttctctagcctgg

SEQ ID NO: 185 - RNA, 16 nt, synthetic construct
  source 1..16: mol_type = other RNA
ctggcggatctcaaca

SEQ ID NO: 186 - RNA, 21 nt, synthetic construct
  source 1..21: mol_type = other RNA
tgttgagatccgccagcgacg

SEQ ID NO: 187 - RNA, 16 nt, synthetic construct
  source 1..16: mol_type = other RNA
agcttcttattggtga

SEQ ID NO: 188 - RNA, 21 nt, synthetic construct
  source 1..21: mol_type = other RNA
tcaccaataagaagctcatcc

SEQ ID NO: 189 - RNA, 16 nt, synthetic construct
  source 1..16: mol_type = other RNA
gcattttaaccacaga

SEQ ID NO: 190 - RNA, 21 nt, synthetic construct
  source 1..21: mol_type = other RNA
tctgtggttaaaatgcatctg

SEQ ID NO: 191 - RNA, 16 nt, synthetic construct
  source 1..16: mol_type = other RNA
tccagatgcattttaa

SEQ ID NO: 192 - RNA, 21 nt, synthetic construct
  source 1..21: mol_type = other RNA
ttaaaatgcatctggaacaag

SEQ ID NO: 193 - RNA, 16 nt, synthetic construct
  source 1..16: mol_type = other RNA
ttccagatgcatttta

SEQ ID NO: 194 - RNA, 21 nt, synthetic construct
  source 1..21: mol_type = other RNA
taaaatgcatctggaacaagc

SEQ ID NO: 195 - RNA, 16 nt, synthetic construct
  source 1..16: mol_type = other RNA
gttccagatgcattta

SEQ ID NO: 196 - RNA, 21 nt, synthetic construct
  source 1..21: mol_type = other RNA
taaatgcatctggaacaagcc

SEQ ID NO: 197 - RNA, 16 nt, synthetic construct
  source 1..16: mol_type = other RNA
tgttccagatgcatta

SEQ ID NO: 198 - RNA, 21 nt, synthetic construct
  source 1..21: mol_type = other RNA
taatgcatctggaacaagcca

SEQ ID NO: 199 - RNA, 16 nt, synthetic construct
  source 1..16: mol_type = other RNA
ttgttccagatgcata

SEQ ID NO: 200 - RNA, 21 nt, synthetic construct
  source 1..21: mol_type = other RNA
tatgcatctggaacaagccat

SEQ ID NO: 201 - RNA, 16 nt, synthetic construct
  source 1..16: mol_type = other RNA
gtgtcatgagcaggaa

SEQ ID NO: 202 - RNA, 21 nt, synthetic construct
  source 1..21: mol_type = other RNA
ttcctgctcatgacaccggtg

SEQ ID NO: 203 - RNA, 16 nt, synthetic construct
  source 1..16: mol_type = other RNA
ctgctgggccagtaaa

SEQ ID NO: 204 - RNA, 21 nt, synthetic construct
  source 1..21: mol_type = other RNA
tttactggcccagcaggtaca

SEQ ID NO: 205 - RNA, 16 nt, synthetic construct
  source 1..16: mol_type = other RNA
cctgctgggccagtaa

SEQ ID NO: 206 - RNA, 21 nt, synthetic construct
  source 1..21: mol_type = other RNA
ttactggcccagcaggtacac

SEQ ID NO: 207 - RNA, 16 nt, synthetic construct
  source 1..16: mol_type = other RNA
cccagggaccatcaaa

SEQ ID NO: 208 - RNA, 21 nt, synthetic construct
  source 1..21: mol_type = other RNA
tttgatggtccctgggttttc

SEQ ID NO: 209 - RNA, 16 nt, synthetic construct
  source 1..16: mol_type = other RNA
acccagggaccatcaa

SEQ ID NO: 210 - RNA, 21 nt, synthetic construct
  source 1..21: mol_type = other RNA
ttgatggtccctgggttttcc

SEQ ID NO: 211 - RNA, 16 nt, synthetic construct
  source 1..16: mol_type = other RNA
ggcagtattttgtgca

SEQ ID NO: 212 - RNA, 21 nt, synthetic construct
  source 1..21: mol_type = other RNA
tgcacaaaatactgcccaaag

SEQ ID NO: 213 - RNA, 16 nt, synthetic construct
  source 1..16: mol_type = other RNA
ctttgggcagtattta

SEQ ID NO: 214 - RNA, 21 nt, synthetic construct
  source 1..21: mol_type = other RNA
taaatactgcccaaagagtgg

SEQ ID NO: 215 - RNA, 16 nt, synthetic construct
  source 1..16: mol_type = other RNA
tctttgggcagtatta

SEQ ID NO: 216 - RNA, 21 nt, synthetic construct
  source 1..21: mol_type = other RNA
taatactgcccaaagagtggt

SEQ ID NO: 217 - RNA, 16 nt, synthetic construct
  source 1..16: mol_type = other RNA
ctctttgggcagtata

SEQ ID NO: 218 - RNA, 21 nt, synthetic construct
  source 1..21: mol_type = other RNA
tatactgcccaaagagtggtg

SEQ ID NO: 219 - RNA, 16 nt, synthetic construct
  source 1..16: mol_type = other RNA
actctttgggcagtaa

SEQ ID NO: 220 - RNA, 21 nt, synthetic construct
  source 1..21: mol_type = other RNA
ttactgcccaaagagtggtga

SEQ ID NO: 221 - RNA, 16 nt, synthetic construct
  source 1..16: mol_type = other RNA
cactctttgggcagta

SEQ ID NO: 222 - RNA, 21 nt, synthetic construct
  source 1..21: mol_type = other RNA
tactgcccaaagagtggtgat

SEQ ID NO: 223 - RNA, 16 nt, synthetic construct
  source 1..16: mol_type = other RNA
ccactctttgggcaga

SEQ ID NO: 224 - RNA, 21 nt, synthetic construct
  source 1..21: mol_type = other RNA
tctgcccaaagagtggtgatt

SEQ ID NO: 225 - RNA, 16 nt, synthetic construct
  source 1..16: mol_type = other RNA
ggaaaatcaccactca

SEQ ID NO: 226 - RNA, 21 nt, synthetic construct
  source 1..21: mol_type = other RNA
tgagtggtgattttccatata

SEQ ID NO: 227 - RNA, 16 nt, synthetic construct
  source 1..16: mol_type = other RNA
cgaaagttatatggaa

SEQ ID NO: 228 - RNA, 21 nt, synthetic construct
  source 1..21: mol_type = other RNA
ttccatataactttcgttctg

SEQ ID NO: 229 - RNA, 16 nt, synthetic construct
  source 1..16: mol_type = other RNA
cagaacgaaagttata

SEQ ID NO: 230 - RNA, 21 nt, synthetic construct
  source 1..21: mol_type = other RNA
tataactttcgttctgaaggg

SEQ ID NO: 231 - RNA, 16 nt, synthetic construct
  source 1..16: mol_type = other RNA
tcagaacgaaagttaa

SEQ ID NO: 232 - RNA, 21 nt, synthetic construct
  source 1..21: mol_type = other RNA
ttaactttcgttctgaagggt

SEQ ID NO: 233 - RNA, 16 nt, synthetic construct
  source 1..16: mol_type = other RNA
ttcagaacgaaagtta

SEQ ID NO: 234 - RNA, 21 nt, synthetic construct
  source 1..21: mol_type = other RNA
taactttcgttctgaagggtc

SEQ ID NO: 235 - RNA, 16 nt, synthetic construct
  source 1..16: mol_type = other RNA
ccttcagaacgaaaga

SEQ ID NO: 236 - RNA, 21 nt, synthetic construct
  source 1..21: mol_type = other RNA
tctttcgttctgaagggtcac

SEQ ID NO: 237 - RNA, 16 nt, synthetic construct
  source 1..16: mol_type = other RNA
acccttcagaacgaaa

SEQ ID NO: 238 - RNA, 21 nt, synthetic construct
  source 1..21: mol_type = other RNA
tttcgttctgaagggtcacac

SEQ ID NO: 239 - RNA, 16 nt, synthetic construct
  source 1..16: mol_type = other RNA
gacccttcagaacgaa

SEQ ID NO: 240 - RNA, 21 nt, synthetic construct
  source 1..21: mol_type = other RNA
ttcgttctgaagggtcacact

SEQ ID NO: 241 - RNA, 16 nt, synthetic construct
  source 1..16: mol_type = other RNA
ggaaccgctggaaaca

SEQ ID NO: 242 - RNA, 21 nt, synthetic construct
  source 1..21: mol_type = other RNA
tgtttccagcggttccttcct

SEQ ID NO: 243 - RNA, 16 nt, synthetic construct
  source 1..16: mol_type = other RNA
tcctggaatattagaa

SEQ ID NO: 244 - RNA, 21 nt, synthetic construct
  source 1..21: mol_type = other RNA
ttctaatattccaggacatac

SEQ ID NO: 245 - RNA, 16 nt, synthetic construct
  source 1..16: mol_type = other RNA
gtcctggaatattaga

SEQ ID NO: 246 - RNA, 21 nt, synthetic construct
  source 1..21: mol_type = other RNA
tctaatattccaggacatacg

SEQ ID NO: 247 - RNA, 16 nt, synthetic construct
  source 1..16: mol_type = other RNA
atgtcctggaatatta

SEQ ID NO: 248 - RNA, 21 nt, synthetic construct
  source 1..21: mol_type = other RNA
taatattccaggacatacggt

SEQ ID NO: 249 - RNA, 16 nt, synthetic construct
  source 1..16: mol_type = other RNA
gtatgtcctggaataa

SEQ ID NO: 250 - RNA, 21 nt, synthetic construct
  source 1..21: mol_type = other RNA
ttattccaggacatacggttc

SEQ ID NO: 251 - RNA, 16 nt, synthetic construct
  source 1..16: mol_type = other RNA
cgtatgtcctggaata

SEQ ID NO: 252 - RNA, 21 nt, synthetic construct
  source 1..21: mol_type = other RNA
tattccaggacatacggttcc

SEQ ID NO: 253 - RNA, 16 nt, synthetic construct
  source 1..16: mol_type = other RNA
ccgtatgtcctggaaa

SEQ ID NO: 254 - RNA, 21 nt, synthetic construct
  source 1..21: mol_type = other RNA
tttccaggacatacggttccc

SEQ ID NO: 255 - RNA, 16 nt, synthetic construct
  source 1..16: mol_type = other RNA
accgtatgtcctggaa

SEQ ID NO: 256 - RNA, 21 nt, synthetic construct
  source 1..21: mol_type = other RNA
ttccaggacatacggttccca

SEQ ID NO: 257 - RNA, 16 nt, synthetic construct
  source 1..16: mol_type = other RNA
cagaactgagacctca

SEQ ID NO: 258 - RNA, 21 nt, synthetic construct
  source 1..21: mol_type = other RNA
tgaggtctcagttctgaaaca

SEQ ID NO: 259 - RNA, 16 nt, synthetic construct
  source 1..16: mol_type = other RNA
ggtgtttcagaactga

SEQ ID NO: 260 - RNA, 21 nt, synthetic construct
  source 1..21: mol_type = other RNA
tcagttctgaaacaccatgct

SEQ ID NO: 261 - RNA, 16 nt, synthetic construct
  source 1..16: mol_type = other RNA
gcatggtgtttcagaa

SEQ ID NO: 262 - RNA, 21 nt, synthetic construct
  source 1..21: mol_type = other RNA
ttctgaaacaccatgcttcaa

SEQ ID NO: 263 - RNA, 16 nt, synthetic construct
  source 1..16: mol_type = other RNA
agcatggtgtttcaga

SEQ ID NO: 264 - RNA, 21 nt, synthetic construct
  source 1..21: mol_type = other RNA
tctgaaacaccatgcttcaag

SEQ ID NO: 265 - RNA, 16 nt, synthetic construct
  source 1..16: mol_type = other RNA
ttgaagcatggtgtta

SEQ ID NO: 266 - RNA, 21 nt, synthetic construct
  source 1..21: mol_type = other RNA
taacaccatgcttcaagtgtt

SEQ ID NO: 267 - RNA, 16 nt, synthetic construct
  source 1..16: mol_type = other RNA
ctcaaaaatgacaaca

SEQ ID NO: 268 - RNA, 21 nt, synthetic construct
  source 1..21: mol_type = other RNA
tgttgtcatttttgagaacat

SEQ ID NO: 269 - RNA, 16 nt, synthetic construct
  source 1..16: mol_type = other RNA
ctctacattttcttta

SEQ ID NO: 270 - RNA, 21 nt, synthetic construct
  source 1..21: mol_type = other RNA
taaagaaaatgtagaggtctc

SEQ ID NO: 271 - RNA, 16 nt, synthetic construct
  source 1..16: mol_type = other RNA
cgtcttttggacttca

SEQ ID NO: 272 - RNA, 21 nt, synthetic construct
  source 1..21: mol_type = other RNA
tgaagtccaaaagacgaaaaa

SEQ ID NO: 273 - RNA, 16 nt, synthetic construct
  source 1..16: mol_type = other RNA
gcttcaatgtcccaga

SEQ ID NO: 274 - RNA, 21 nt, synthetic construct
  source 1..21: mol_type = other RNA
tctgggacattgaagcattga

SEQ ID NO: 275 - RNA, 16 nt, synthetic construct
  source 1..16: mol_type = other RNA
ctcaatgcttcaatga

SEQ ID NO: 276 - RNA, 21 nt, synthetic construct
  source 1..21: mol_type = other RNA
tcattgaagcattgagacacc

SEQ ID NO: 277 - RNA, 16 nt, synthetic construct
  source 1..16: mol_type = other RNA
gtctcaatgcttcaaa

SEQ ID NO: 278 - RNA, 21 nt, synthetic construct
  source 1..21: mol_type = other RNA
tttgaagcattgagacaccag

SEQ ID NO: 279 - RNA, 16 nt, synthetic construct
  source 1..16: mol_type = other RNA
gtgtctcaatgcttca

SEQ ID NO: 280 - RNA, 21 nt, synthetic construct
  source 1..21: mol_type = other RNA
tgaagcattgagacaccagaa

SEQ ID NO: 281 - RNA, 16 nt, synthetic construct
  source 1..16: mol_type = other RNA
tggtgtctcaatgcta

SEQ ID NO: 282 - RNA, 21 nt, synthetic construct
  source 1..21: mol_type = other RNA
tagcattgagacaccagaagt

SEQ ID NO: 283 - RNA, 16 nt, synthetic construct
  source 1..16: mol_type = other RNA
caggattctgaaaaca

SEQ ID NO: 284 - RNA, 21 nt, synthetic construct
  source 1..21: mol_type = other RNA
tgttttcagaatcctgtcttg

SEQ ID NO: 285 - RNA, 16 nt, synthetic construct
  source 1..16: mol_type = other RNA
gacaggattctgaaaa

SEQ ID NO: 286 - RNA, 21 nt, synthetic construct
  source 1..21: mol_type = other RNA
ttttcagaatcctgtcttgtc

SEQ ID NO: 287 - RNA, 16 nt, synthetic construct
  source 1..16: mol_type = other RNA
agacaggattctgaaa

SEQ ID NO: 288 - RNA, 21 nt, synthetic construct
  source 1..21: mol_type = other RNA
tttcagaatcctgtcttgtca

SEQ ID NO: 289 - RNA, 16 nt, synthetic construct
  source 1..16: mol_type = other RNA
gacaagacaggattca

SEQ ID NO: 290 - RNA, 21 nt, synthetic construct
  source 1..21: mol_type = other RNA
tgaatcctgtcttgtcattta

SEQ ID NO: 291 - RNA, 16 nt, synthetic construct
  source 1..16: mol_type = other RNA
atgacaagacaggata

SEQ ID NO: 292 - RNA, 21 nt, synthetic construct
  source 1..21: mol_type = other RNA
tatcctgtcttgtcatttaag

SEQ ID NO: 293 - RNA, 16 nt, synthetic construct
  source 1..16: mol_type = other RNA
ccgtttaactgattaa

SEQ ID NO: 294 - RNA, 21 nt, synthetic construct
  source 1..21: mol_type = other RNA
ttaatcagttaaacggggagt

SEQ ID NO: 295 - RNA, 16 nt, synthetic construct
  source 1..16: mol_type = other RNA
cccgtttaactgatta

SEQ ID NO: 296 - RNA, 21 nt, synthetic construct
  source 1..21: mol_type = other RNA
taatcagttaaacggggagtt

SEQ ID NO: 297 - RNA, 16 nt, synthetic construct
  source 1..16: mol_type = other RNA
ccccgtttaactgata

SEQ ID NO: 298 - RNA, 21 nt, synthetic construct
  source 1..21: mol_type = other RNA
tatcagttaaacggggagttt

SEQ ID NO: 299 - RNA, 16 nt, synthetic construct
  source 1..16: mol_type = other RNA
cgtttatctaccaaga

SEQ ID NO: 300 - RNA, 21 nt, synthetic construct
  source 1..21: mol_type = other RNA
tcttggtagataaacggagaa

SEQ ID NO: 301 - RNA, 16 nt, synthetic construct
  source 1..16: mol_type = other RNA
tccgtttatctaccaa

SEQ ID NO: 302 - RNA, 21 nt, synthetic construct
  source 1..21: mol_type = other RNA
ttggtagataaacggagaagc

SEQ ID NO: 303 - RNA, 16 nt, synthetic construct
  source 1..16: mol_type = other RNA
tcctgtcactaccaca

SEQ ID NO: 304 - RNA, 21 nt, synthetic construct
  source 1..21: mol_type = other RNA
tgtggtagtgacaggatgcaa

SEQ ID NO: 305 - RNA, 16 nt, synthetic construct
  source 1..16: mol_type = other RNA
gagaaagaggaagaga

SEQ ID NO: 306 - RNA, 21 nt, synthetic construct
  source 1..21: mol_type = other RNA
tctcttcctctttctcttctt

SEQ ID NO: 307 - RNA, 16 nt, synthetic construct
  source 1..16: mol_type = other RNA
gagaagaagagaaaga

SEQ ID NO: 308 - RNA, 21 nt, synthetic construct
  source 1..21: mol_type = other RNA
tctttctcttcttctctttct

SEQ ID NO: 309 - RNA, 16 nt, synthetic construct
  source 1..16: mol_type = other RNA
aagagaagaagagaaa

SEQ ID NO: 310 - RNA, 21 nt, synthetic construct
  source 1..21: mol_type = other RNA
tttctcttcttctctttctct

SEQ ID NO: 311 - RNA, 16 nt, synthetic construct
  source 1..16: mol_type = other RNA
gagaaagagaagaaga

SEQ ID NO: 312 - RNA, 21 nt, synthetic construct
  source 1..21: mol_type = other RNA
tcttcttctctttctctaacg

SEQ ID NO: 313 - RNA, 16 nt, synthetic construct
  source 1..16: mol_type = other RNA
tacgcaatgaaaatta

SEQ ID NO: 314 - RNA, 21 nt, synthetic construct
  source 1..21: mol_type = other RNA
taattttcattgcgtacctca

SEQ ID NO: 315 - RNA, 16 nt, synthetic construct
  source 1..16: mol_type = other RNA
gtacgcaatgaaaata

SEQ ID NO: 316 - RNA, 21 nt, synthetic construct
  source 1..21: mol_type = other RNA
tattttcattgcgtacctcat

SEQ ID NO: 317 - RNA, 16 nt, synthetic construct
  source 1..16: mol_type = other RNA
caaatatggctggaaa

SEQ ID NO: 318 - RNA, 21 nt, synthetic construct
  source 1..21: mol_type = other RNA
tttccagccatatttggggtg

SEQ ID NO: 319 - RNA, 16 nt, synthetic construct
  source 1..16: mol_type = other RNA
cccaaatatggctgga

SEQ ID NO: 320 - RNA, 21 nt, synthetic construct
  source 1..21: mol_type = other RNA
tccagccatatttggggtgca

SEQ ID NO: 321 - RNA, 16 nt, synthetic construct
  source 1..16: mol_type = other RNA
cttttgaaatggcata

SEQ ID NO: 322 - RNA, 21 nt, synthetic construct
  source 1..21: mol_type = other RNA
tatgccatttcaaaagctagc

SEQ ID NO: 323 - RNA, 16 nt, synthetic construct
  source 1..16: mol_type = other RNA
gcttttgaaatggcaa

SEQ ID NO: 324 - RNA, 21 nt, synthetic construct
  source 1..21: mol_type = other RNA
ttgccatttcaaaagctagcc

SEQ ID NO: 325 - RNA, 16 nt, synthetic construct
  source 1..16: mol_type = other RNA
ggctagcttttgaaaa

SEQ ID NO: 326 - RNA, 21 nt, synthetic construct
  source 1..21: mol_type = other RNA
ttttcaaaagctagcccgggg

SEQ ID NO: 327 - RNA, 16 nt, synthetic construct
  source 1..16: mol_type = other RNA
gggctagcttttgaaa

SEQ ID NO: 328 - RNA, 21 nt, synthetic construct
  source 1..21: mol_type = other RNA
tttcaaaagctagcccggggc

SEQ ID NO: 329 - RNA, 16 nt, synthetic construct
  source 1..16: mol_type = other RNA
cgggctagcttttgaa

SEQ ID NO: 330 - RNA, 21 nt, synthetic construct
  source 1..21: mol_type = other RNA
ttcaaaagctagcccggggct

SEQ ID NO: 331 - RNA, 16 nt, synthetic construct
  source 1..16: mol_type = other RNA
ccgggctagcttttga

SEQ ID NO: 332 - RNA, 21 nt, synthetic construct
  source 1..21: mol_type = other RNA
tcaaaagctagcccggggctt

SEQ ID NO: 333 - RNA, 16 nt, synthetic construct
  source 1..16: mol_type = other RNA
ccccgggctagcttta

SEQ ID NO: 334 - RNA, 21 nt, synthetic construct
  source 1..21: mol_type = other RNA
taaagctagcccggggcttga

SEQ ID NO: 335 - RNA, 16 nt, synthetic construct
  source 1..16: mol_type = other RNA
gccccgggctagctta

SEQ ID NO: 336 - RNA, 21 nt, synthetic construct
  source 1..21: mol_type = other RNA
taagctagcccggggcttgag

SEQ ID NO: 337 - RNA, 16 nt, synthetic construct
  source 1..16: mol_type = other RNA
agccccgggctagcta

SEQ ID NO: 338 - RNA, 21 nt, synthetic construct
  source 1..21: mol_type = other RNA
tagctagcccggggcttgaga

SEQ ID NO: 339 - RNA, 16 nt, synthetic construct
  source 1..16: mol_type = other RNA
ctcaagccccgggcta

SEQ ID NO: 340 - RNA, 21 nt, synthetic construct
  source 1..21: mol_type = other RNA
tagcccggggcttgagaagaa

SEQ ID NO: 341 - RNA, 16 nt, synthetic construct
  source 1..16: mol_type = other RNA
accttcaggaagcaca

SEQ ID NO: 342 - RNA, 21 nt, synthetic construct
  source 1..21: mol_type = other RNA
tgtgcttcctgaaggtcacct

SEQ ID NO: 343 - RNA, 16 nt, synthetic construct
  source 1..16: mol_type = other RNA
aggtgaccttcaggaa

SEQ ID NO: 344 - RNA, 21 nt, synthetic construct
  source 1..21: mol_type = other RNA
ttcctgaaggtcacctcagtc

SEQ ID NO: 345 - RNA, 16 nt, synthetic construct
  source 1..16: mol_type = other RNA
ccatagatctggatca

SEQ ID NO: 346 - RNA, 21 nt, synthetic construct
  source 1..21: mol_type = other RNA
tgatccagatctatggaaaat

SEQ ID NO: 347 - RNA, 16 nt, synthetic construct
  source 1..16: mol_type = other RNA
ctgcagatattaatta

SEQ ID NO: 348 - RNA, 21 nt, synthetic construct
  source 1..21: mol_type = other RNA
taattaatatctgcagtgctt

SEQ ID NO: 349 - RNA, 16 nt, synthetic construct
  source 1..16: mol_type = other RNA
actgcagatattaata

SEQ ID NO: 350 - RNA, 21 nt, synthetic construct
  source 1..21: mol_type = other RNA
tattaatatctgcagtgcttc

SEQ ID NO: 351 - RNA, 16 nt, synthetic construct
  source 1..16: mol_type = other RNA
cattggatttcctaaa

SEQ ID NO: 352 - RNA, 21 nt, synthetic construct
  source 1..21: mol_type = other RNA
tttaggaaatccaatgctgtc

SEQ ID NO: 353 - RNA, 16 nt, synthetic construct
  source 1..16: mol_type = other RNA
gcattggatttcctaa

SEQ ID NO: 354 - RNA, 21 nt, synthetic construct
  source 1..21: mol_type = other RNA
ttaggaaatccaatgctgtct

SEQ ID NO: 355 - RNA, 16 nt, synthetic construct
  source 1..16: mol_type = other RNA
agcattggatttccta

SEQ ID NO: 356 - RNA, 21 nt, synthetic construct
  source 1..21: mol_type = other RNA
taggaaatccaatgctgtctg

SEQ ID NO: 357 - RNA, 16 nt, synthetic construct
  source 1..16: mol_type = other RNA
agacagcattggatta

SEQ ID NO: 358 - RNA, 21 nt, synthetic construct
  source 1..21: mol_type = other RNA
taatccaatgctgtctgagaa

SEQ ID NO: 359 - RNA, 16 nt, synthetic construct
  source 1..16: mol_type = other RNA
cagacagcattggata

SEQ ID NO: 360 - RNA, 21 nt, synthetic construct
  source 1..21: mol_type = other RNA
tatccaatgctgtctgagaag

SEQ ID NO: 361 - RNA, 16 nt, synthetic construct
  source 1..16: mol_type = other RNA
gcttctcagacagcaa

SEQ ID NO: 362 - RNA, 21 nt, synthetic construct
  source 1..21: mol_type = other RNA
ttgctgtctgagaagcagcag

SEQ ID NO: 363 - RNA, 16 nt, synthetic construct
  source 1..16: mol_type = other RNA
tgctgcttctcagaca

SEQ ID NO: 364 - RNA, 21 nt, synthetic construct
  source 1..21: mol_type = other RNA
tgtctgagaagcagcagggcc

SEQ ID NO: 365 - RNA, 16 nt, synthetic construct
  source 1..16: mol_type = other RNA
cctgctgcttctcaga

SEQ ID NO: 366 - RNA, 21 nt, synthetic construct
  source 1..21: mol_type = other RNA
tctgagaagcagcagggccag

SEQ ID NO: 367 - RNA, 16 nt, synthetic construct
  source 1..16: mol_type = other RNA
aggatggttgtgtaga

SEQ ID NO: 368 - RNA, 21 nt, synthetic construct
  source 1..21: mol_type = other RNA
tctacacaaccatcctcctga

SEQ ID NO: 369 - RNA, 16 nt, synthetic construct
  source 1..16: mol_type = other RNA
ctggatccttgccata

SEQ ID NO: 370 - RNA, 21 nt, synthetic construct
  source 1..21: mol_type = other RNA
tatggcaaggatccaggggtc

SEQ ID NO: 371 - RNA, 16 nt, synthetic construct
  source 1..16: mol_type = other RNA
cctggatccttgccaa

SEQ ID NO: 372 - RNA, 21 nt, synthetic construct
  source 1..21: mol_type = other RNA
ttggcaaggatccaggggtcc

SEQ ID NO: 373 - RNA, 16 nt, synthetic construct
  source 1..16: mol_type = other RNA
ccctggatccttgcca

SEQ ID NO: 374 - RNA, 21 nt, synthetic construct
  source 1..21: mol_type = other RNA
tggcaaggatccaggggtcct

SEQ ID NO: 375 - RNA, 16 nt, synthetic construct
  source 1..16: mol_type = other RNA
ggacccctggatccta

SEQ ID NO: 376 - RNA, 21 nt, synthetic construct
  source 1..21: mol_type = other RNA
taggatccaggggtcctccat

SEQ ID NO: 377 - RNA, 16 nt, synthetic construct
  source 1..16: mol_type = other RNA
tggaggacccctggaa

SEQ ID NO: 378 - RNA, 21 nt, synthetic construct
  source 1..21: mol_type = other RNA
ttccaggggtcctccatgact

SEQ ID NO: 379 - RNA, 16 nt, synthetic construct
  source 1..16: mol_type = other RNA
tgctccttctccagta

SEQ ID NO: 380 - RNA, 21 nt, synthetic construct
  source 1..21: mol_type = other RNA
tactggagaaggagcactccg

SEQ ID NO: 381 - RNA, 16 nt, synthetic construct
  source 1..16: mol_type = other RNA
gtgctccttctccaga

SEQ ID NO: 382 - RNA, 21 nt, synthetic construct
  source 1..21: mol_type = other RNA
tctggagaaggagcactccgt

SEQ ID NO: 383 - RNA, 16 nt, synthetic construct
  source 1..16: mol_type = other RNA
acggagtgctccttca

SEQ ID NO: 384 - RNA, 21 nt, synthetic construct
  source 1..21: mol_type = other RNA
tgaaggagcactccgtcatta

SEQ ID NO: 385 - RNA, 16 nt, synthetic construct
  source 1..16: mol_type = other RNA
tgaaaaagttctgaaa

SEQ ID NO: 386 - RNA, 21 nt, synthetic construct
  source 1..21: mol_type = other RNA
tttcagaactttttcacccgg

SEQ ID NO: 387 - RNA, 16 nt, synthetic construct
  source 1..16: mol_type = other RNA
gtgaaaaagttctgaa

SEQ ID NO: 388 - RNA, 21 nt, synthetic construct
  source 1..21: mol_type = other RNA
ttcagaactttttcacccgga

SEQ ID NO: 389 - RNA, 16 nt, synthetic construct
  source 1..16: mol_type = other RNA
ggtgaaaaagttctga

SEQ ID NO: 390 - RNA, 21 nt, synthetic construct
  source 1..21: mol_type = other RNA
tcagaactttttcacccggaa

SEQ ID NO: 391 - RNA, 16 nt, synthetic construct
  source 1..16: mol_type = other RNA
cgggtgaaaaagttca

SEQ ID NO: 392 - RNA, 21 nt, synthetic construct
  source 1..21: mol_type = other RNA
tgaactttttcacccggaact

SEQ ID NO: 393 - RNA, 16 nt, synthetic construct
  source 1..16: mol_type = other RNA
tccgggtgaaaaagta

SEQ ID NO: 394 - RNA, 21 nt, synthetic construct
  source 1..21: mol_type = other RNA
tactttttcacccggaactgg

SEQ ID NO: 395 - RNA, 16 nt, synthetic construct
  source 1..16: mol_type = other RNA
aagtgattcagtgata

SEQ ID NO: 396 - RNA, 21 nt, synthetic construct
  source 1..21: mol_type = other RNA
tatcactgaatcacttttctt

SEQ ID NO: 397 - RNA, 16 nt, synthetic construct
  source 1..16: mol_type = other RNA
gagaagaaaagtgata

SEQ ID NO: 398 - RNA, 21 nt, synthetic construct
  source 1..21: mol_type = other RNA
tatcacttttcttctcctcca

SEQ ID NO: 399 - RNA, 16 nt, synthetic construct
  source 1..16: mol_type = other RNA
ggagaagaaaagtgaa

SEQ ID NO: 400 - RNA, 21 nt, synthetic construct
  source 1..21: mol_type = other RNA
ttcacttttcttctcctccac

SEQ ID NO: 401 - RNA, 16 nt, synthetic construct
  source 1..16: mol_type = other RNA
ggaggagaagaaaaga

SEQ ID NO: 402 - RNA, 21 nt, synthetic construct
  source 1..21: mol_type = other RNA
tcttttcttctcctccacaga

SEQ ID NO: 403 - RNA, 16 nt, synthetic construct
  source 1..16: mol_type = other RNA
gtggaggagaagaaaa

SEQ ID NO: 404 - RNA, 21 nt, synthetic construct
  source 1..21: mol_type = other RNA
ttttcttctcctccacagaat

SEQ ID NO: 405 - RNA, 16 nt, synthetic construct
  source 1..16: mol_type = other RNA
tgtggaggagaagaaa

SEQ ID NO: 406 - RNA, 21 nt, synthetic construct
  source 1..21: mol_type = other RNA
tttcttctcctccacagaatt

SEQ ID NO: 407 - RNA, 16 nt, synthetic construct
  source 1..16: mol_type = other RNA
ctgtggaggagaagaa

SEQ ID NO: 408 - RNA, 21 nt, synthetic construct
  source 1..21: mol_type = other RNA
ttcttctcctccacagaattc

SEQ ID NO: 409 - RNA, 16 nt, synthetic construct
  source 1..16: mol_type = other RNA
ggggaaaaggaaagca

SEQ ID NO: 410 - RNA, 21 nt, synthetic construct
  source 1..21: mol_type = other RNA
tgctttccttttcccccttta

SEQ ID NO: 411 - RNA, 16 nt, synthetic construct
  source 1..16: mol_type = other RNA
aagggggaaaaggaaa

SEQ ID NO: 412 - RNA, 21 nt, synthetic construct
  source 1..21: mol_type = other RNA
tttccttttccccctttaaag

SEQ ID NO: 413 - RNA, 16 nt, synthetic construct
  source 1..16: mol_type = other RNA
ctttaaagggggaaaa

SEQ ID NO: 414 - RNA, 21 nt, synthetic construct
  source 1..21: mol_type = other RNA
ttttccccctttaaaggtttt

SEQ ID NO: 415 - RNA, 16 nt, synthetic construct
  source 1..16: mol_type = other RNA
cctttaaagggggaaa

SEQ ID NO: 416 - RNA, 21 nt, synthetic construct
  source 1..21: mol_type = other RNA
tttccccctttaaaggttttc

SEQ ID NO: 417 - RNA, 16 nt, synthetic construct
  source 1..16: mol_type = other RNA
acctttaaagggggaa

SEQ ID NO: 418 - RNA, 21 nt, synthetic construct
  source 1..21: mol_type = other RNA
ttccccctttaaaggttttca

SEQ ID NO: 419 - RNA, 16 nt, synthetic construct
  source 1..16: mol_type = other RNA
tactgaaaacctttaa

SEQ ID NO: 420 - RNA, 21 nt, synthetic construct
  source 1..21: mol_type = other RNA
ttaaaggttttcagtagtcta

SEQ ID NO: 421 - RNA, 16 nt, synthetic construct
  source 1..16: mol_type = other RNA
ctactgaaaaccttta

SEQ ID NO: 422 - RNA, 21 nt, synthetic construct
  source 1..21: mol_type = other RNA
taaaggttttcagtagtctat

SEQ ID NO: 423 - RNA, 16 nt, synthetic construct
  source 1..16: mol_type = other RNA
actactgaaaacctta

SEQ ID NO: 424 - RNA, 21 nt, synthetic construct
  source 1..21: mol_type = other RNA
taaggttttcagtagtctatc

SEQ ID NO: 425 - RNA, 16 nt, synthetic construct
  source 1..16: mol_type = other RNA
gactactgaaaaccta

SEQ ID NO: 426 - RNA, 21 nt, synthetic construct
  source 1..21: mol_type = other RNA
taggttttcagtagtctatct

SEQ ID NO: 427 - RNA, 16 nt, synthetic construct
  source 1..16: mol_type = other RNA
ttgtttaaaacccaaa

SEQ ID NO: 428 - RNA, 21 nt, synthetic construct
  source 1..21: mol_type = other RNA
tttgggttttaaacaactgac

SEQ ID NO: 429 - RNA, 16 nt, synthetic construct
  source 1..16: mol_type = other RNA
catatgtcagttgtta

SEQ ID NO: 430 - RNA, 21 nt, synthetic construct
  source 1..21: mol_type = other RNA
taacaactgacatatgctttc

SEQ ID NO: 431 - RNA, 16 nt, synthetic construct
  source 1..16: mol_type = other RNA
gcatatgtcagttgta

SEQ ID NO: 432 - RNA, 21 nt, synthetic construct
  source 1..21: mol_type = other RNA
tacaactgacatatgctttcc

SEQ ID NO: 433 - RNA, 16 nt, synthetic construct
  source 1..16: mol_type = other RNA
agcatatgtcagttga

SEQ ID NO: 434 - RNA, 21 nt, synthetic construct
  source 1..21: mol_type = other RNA
tcaactgacatatgctttcct

SEQ ID NO: 435 - RNA, 16 nt, synthetic construct
  source 1..16: mol_type = other RNA
ccattttgtcctttga

SEQ ID NO: 436 - RNA, 21 nt, synthetic construct
  source 1..21: mol_type = other RNA
tcaaaggacaaaatggcaata

SEQ ID NO: 437 - RNA, 16 nt, synthetic construct
  source 1..16: mol_type = other RNA
tgccattttgtcctta

SEQ ID NO: 438 - RNA, 21 nt, synthetic construct
  source 1..21: mol_type = other RNA
taaggacaaaatggcaataaa

SEQ ID NO: 439 - RNA, 16 nt, synthetic construct
  source 1..16: mol_type = other RNA
agatctgatgaagtaa

SEQ ID NO: 440 - RNA, 21 nt, synthetic construct
  source 1..21: mol_type = other RNA
ttacttcatcagatcttagag

SEQ ID NO: 441 - RNA, 16 nt, synthetic construct
  source 1..16: mol_type = other RNA
ctctaagatctgatga

SEQ ID NO: 442 - RNA, 21 nt, synthetic construct
  source 1..21: mol_type = other RNA
tcatcagatcttagagttata

SEQ ID NO: 443 - RNA, 16 nt, synthetic construct
  source 1..16: mol_type = other RNA
ggaagttgactaaaca

SEQ ID NO: 444 - RNA, 21 nt, synthetic construct
  source 1..21: mol_type = other RNA
tgtttagtcaacttcccaata

SEQ ID NO: 445 - RNA, 16 nt, synthetic construct
  source 1..16: mol_type = other RNA
tgggaagttgactaaa

SEQ ID NO: 446 - RNA, 21 nt, synthetic construct
  source 1..21: mol_type = other RNA
tttagtcaacttcccaatata

SEQ ID NO: 447 - RNA, 16 nt, synthetic construct
  source 1..16: mol_type = other RNA
ttgggaagttgactaa

SEQ ID NO: 448 - RNA, 21 nt, synthetic construct
  source 1..21: mol_type = other RNA
ttagtcaacttcccaatataa

SEQ ID NO: 449 - RNA, 16 nt, synthetic construct
  source 1..16: mol_type = other RNA
ctactttgactagtta

SEQ ID NO: 450 - RNA, 21 nt, synthetic construct
  source 1..21: mol_type = other RNA
taactagtcaaagtagcttcc

SEQ ID NO: 451 - RNA, 16 nt, synthetic construct
  source 1..16: mol_type = other RNA
gctactttgactagta

SEQ ID NO: 452 - RNA, 21 nt, synthetic construct
  source 1..21: mol_type = other RNA
tactagtcaaagtagcttcca

SEQ ID NO: 453 - RNA, 16 nt, synthetic construct
  source 1..16: mol_type = other RNA
agctactttgactaga

SEQ ID NO: 454 - RNA, 21 nt, synthetic construct
  source 1..21: mol_type = other RNA
tctagtcaaagtagcttccat

SEQ ID NO: 455 - RNA, 16 nt, synthetic construct
  source 1..16: mol_type = other RNA
ggaagctactttgaca

SEQ ID NO: 456 - RNA, 21 nt, synthetic construct
  source 1..21: mol_type = other RNA
tgtcaaagtagcttccattta

SEQ ID NO: 457 - RNA, 16 nt, synthetic construct
  source 1..16: mol_type = other RNA
gcctggtcctgattta

SEQ ID NO: 458 - RNA, 21 nt, synthetic construct
  source 1..21: mol_type = other RNA
taaatcaggaccaggcgaggt

SEQ ID NO: 459 - RNA, 16 nt, synthetic construct
  source 1..16: mol_type = other RNA
cgcctggtcctgatta

SEQ ID NO: 460 - RNA, 21 nt, synthetic construct
  source 1..21: mol_type = other RNA
taatcaggaccaggcgaggtt

SEQ ID NO: 461 - RNA, 16 nt, synthetic construct
  source 1..16: mol_type = other RNA
tcgcctggtcctgata

SEQ ID NO: 462 - RNA, 21 nt, synthetic construct
  source 1..21: mol_type = other RNA
tatcaggaccaggcgaggttc

SEQ ID NO: 463 - RNA, 16 nt, synthetic construct
  source 1..16: mol_type = other RNA
ctgactctcagtgcaa

SEQ ID NO: 464 - RNA, 21 nt, synthetic construct
  source 1..21: mol_type = other RNA
ttgcactgagagtcagggtgt

SEQ ID NO: 465 - RNA, 16 nt, synthetic construct
  source 1..16: mol_type = other RNA
cctgactctcagtgca

SEQ ID NO: 466 - RNA, 21 nt, synthetic construct
  source 1..21: mol_type = other RNA
tgcactgagagtcagggtgtc

SEQ ID NO: 467 - RNA, 16 nt, synthetic construct
  source 1..16: mol_type = other RNA
caccctgactctcaga

SEQ ID NO: 468 - RNA, 21 nt, synthetic construct
  source 1..21: mol_type = other RNA
tctgagagtcagggtgtcacc

SEQ ID NO: 469 - RNA, 16 nt, synthetic construct
  source 1..16: mol_type = other RNA
gtgacaccctgactca

SEQ ID NO: 470 - RNA, 21 nt, synthetic construct
  source 1..21: mol_type = other RNA
tgagtcagggtgtcaccatcg

SEQ ID NO: 471 - RNA, 16 nt, synthetic construct
  source 1..16: mol_type = other RNA
agattgcttactcaga

SEQ ID NO: 472 - RNA, 21 nt, synthetic construct
  source 1..21: mol_type = other RNA
tctgagtaagcaatctggtcc

SEQ ID NO: 473 - RNA, 16 nt, synthetic construct
  source 1..16: mol_type = other RNA
tctcaactccaggcta

SEQ ID NO: 474 - RNA, 21 nt, synthetic construct
  source 1..21: mol_type = other RNA
tagcctggagttgagatccgc

SEQ ID NO: 475 - RNA, 16 nt, synthetic construct
  source 1..16: mol_type = other RNA
ggatctcaactccaga

SEQ ID NO: 476 - RNA, 21 nt, synthetic construct
  source 1..21: mol_type = other RNA
tctggagttgagatccgccag

SEQ ID NO: 477 - RNA, 16 nt, synthetic construct
  source 1..16: mol_type = other RNA
cggatctcaactccaa

SEQ ID NO: 478 - RNA, 21 nt, synthetic construct
  source 1..21: mol_type = other RNA
ttggagttgagatccgccagc

SEQ ID NO: 479 - RNA, 16 nt, synthetic construct
  source 1..16: mol_type = other RNA
gcggatctcaactcca

SEQ ID NO: 480 - RNA, 21 nt, synthetic construct
  source 1..21: mol_type = other RNA
tggagttgagatccgccagcg

SEQ ID NO: 481 - RNA, 16 nt, synthetic construct
  source 1..16: mol_type = other RNA
ggcggatctcaactca

SEQ ID NO: 482 - RNA, 21 nt, synthetic construct
  source 1..21: mol_type = other RNA
tgagttgagatccgccagcga

SEQ ID NO: 483 - RNA, 16 nt, synthetic construct
  source 1..16: mol_type = other RNA
agggtgatggcttgta

SEQ ID NO: 484 - RNA, 21 nt, synthetic construct
  source 1..21: mol_type = other RNA
tacaagccatcacccttttca

SEQ ID NO: 485 - RNA, 16 nt, synthetic construct
  source 1..16: mol_type = other RNA
acctgctgggccagta

SEQ ID NO: 486 - RNA, 21 nt, synthetic construct
  source 1..21: mol_type = other RNA
tactggcccagcaggtacaca

SEQ ID NO: 487 - RNA, 16 nt, synthetic construct
  source 1..16: mol_type = other RNA
agagaaagagaagaaa

SEQ ID NO: 488 - RNA, 21 nt, synthetic construct
  source 1..21: mol_type = other RNA
tttcttctctttctctaacga

SEQ ID NO: 489 - RNA, 16 nt, synthetic construct
  source 1..16: mol_type = other RNA
tagagaaagagaagaa

SEQ ID NO: 490 - RNA, 21 nt, synthetic construct
  source 1..21: mol_type = other RNA
ttcttctctttctctaacgag

SEQ ID NO: 491 - RNA, 16 nt, synthetic construct
  source 1..16: mol_type = other RNA
aggagaagaaaagtga

SEQ ID NO: 492 - RNA, 21 nt, synthetic construct
  source 1..21: mol_type = other RNA
tcacttttcttctcctccaca

SEQ ID NO: 493 - RNA, 16 nt, synthetic construct
  source 1..16: mol_type = other RNA
gcagcctacacaaaga

SEQ ID NO: 494 - RNA, 21 nt, synthetic construct
  source 1..21: mol_type = other RNA
tctttgtgtaggctgcactga

SEQ ID NO: 495 - RNA, 16 nt, synthetic construct
  source 1..16: mol_type = other RNA
tgcagcctacacaaaa

SEQ ID NO: 496 - RNA, 21 nt, synthetic construct
  source 1..21: mol_type = other RNA
ttttgtgtaggctgcactgag

SEQ ID NO: 497 - RNA, 16 nt, synthetic construct
  source 1..16: mol_type = other RNA
cagtgcagcctacaca

SEQ ID NO: 498 - RNA, 21 nt, synthetic construct
  source 1..21: mol_type = other RNA
tgtgtaggctgcactgagagt

SEQ ID NO: 499 - RNA, 16 nt, synthetic construct
  source 1..16: mol_type = other RNA
ctcagtgcagcctaca

SEQ ID NO: 500 - RNA, 21 nt, synthetic construct
  source 1..21: mol_type = other RNA
tgtaggctgcactgagagtca

SEQ ID NO: 501 - RNA, 16 nt, synthetic construct
  source 1..16: mol_type = other RNA
tctcagtgcagcctaa

SEQ ID NO: 502 - RNA, 21 nt, synthetic construct
  source 1..21: mol_type = other RNA
ttaggctgcactgagagtcag

SEQ ID NO: 503 - RNA, 16 nt, synthetic construct
  source 1..16: mol_type = other RNA
ctctcagtgcagccta

SEQ ID NO: 504 - RNA, 21 nt, synthetic construct
  source 1..21: mol_type = other RNA
taggctgcactgagagtcagg

SEQ ID NO: 505 - RNA, 16 nt, synthetic construct
  source 1..16: mol_type = other RNA
cctttctgaggcgtca

SEQ ID NO: 506 - RNA, 21 nt, synthetic construct
  source 1..21: mol_type = other RNA
tgacgcctcagaaaggatcaa

SEQ ID NO: 507 - RNA, 16 nt, synthetic construct
  source 1..16: mol_type = other RNA
tcctttctgaggcgta

SEQ ID NO: 508 - RNA, 21 nt, synthetic construct
  source 1..21: mol_type = other RNA
tacgcctcagaaaggatcaag

SEQ ID NO: 509 - RNA, 16 nt, synthetic construct
  source 1..16: mol_type = other RNA
aagaaagttaaagcaa

SEQ ID NO: 510 - RNA, 21 nt, synthetic construct
  source 1..21: mol_type = other RNA
ttgctttaactttcttctcta

SEQ ID NO: 511 - RNA, 16 nt, synthetic construct
  source 1..16: mol_type = other RNA
ggtgacgtggaactga

SEQ ID NO: 512 - RNA, 21 nt, synthetic construct
  source 1..21: mol_type = other RNA
tcagttccacgtcaccaataa

SEQ ID NO: 513 - RNA, 16 nt, synthetic construct
  source 1..16: mol_type = other RNA
tggtgacgtggaacta

SEQ ID NO: 514 - RNA, 21 nt, synthetic construct
  source 1..21: mol_type = other RNA
tagttccacgtcaccaataag

SEQ ID NO: 515 - RNA, 16 nt, synthetic construct
  source 1..16: mol_type = other RNA
cagatgcattttaaca

SEQ ID NO: 516 - RNA, 21 nt, synthetic construct
  source 1..21: mol_type = other RNA
tgttaaaatgcatctggaaca

SEQ ID NO: 517 - RNA, 16 nt, synthetic construct
  source 1..16: mol_type = other RNA
ccatcaaagtgggaga

SEQ ID NO: 518 - RNA, 21 nt, synthetic construct
  source 1..21: mol_type = other RNA
tctcccactttgatggtccct

SEQ ID NO: 519 - RNA, 16 nt, synthetic construct
  source 1..16: mol_type = other RNA
cagggaccatcaaaga

SEQ ID NO: 520 - RNA, 21 nt, synthetic construct
  source 1..21: mol_type = other RNA
tctttgatggtccctgggttt

SEQ ID NO: 521 - RNA, 16 nt, synthetic construct
  source 1..16: mol_type = other RNA
ccagggaccatcaaaa

SEQ ID NO: 522 - RNA, 21 nt, synthetic construct
  source 1..21: mol_type = other RNA
ttttgatggtccctgggtttt

SEQ ID NO: 523 - RNA, 16 nt, synthetic construct
  source 1..16: mol_type = other RNA
tattttgtgctggaaa

SEQ ID NO: 524 - RNA, 21 nt, synthetic construct
  source 1..21: mol_type = other RNA
tttccagcacaaaatactgcc

SEQ ID NO: 525 - RNA, 16 nt, synthetic construct
  source 1..16: mol_type = other RNA
ttgggcagtattttga

SEQ ID NO: 526 - RNA, 21 nt, synthetic construct
  source 1..21: mol_type = other RNA
tcaaaatactgcccaaagagt

SEQ ID NO: 527 - RNA, 16 nt, synthetic construct
  source 1..16: mol_type = other RNA
acgcaatgaaaattaa

SEQ ID NO: 528 - RNA, 21 nt, synthetic construct
  source 1..21: mol_type = other RNA
ttaattttcattgcgtacctc

SEQ ID NO: 529 - RNA, 16 nt, synthetic construct
  source 1..16: mol_type = other RNA
ccaaatatggctggaa

SEQ ID NO: 530 - RNA, 21 nt, synthetic construct
  source 1..21: mol_type = other RNA
ttccagccatatttggggtgc

SEQ ID NO: 531 - RNA, 16 nt, synthetic construct
  source 1..16: mol_type = other RNA
cttctcagacagcata

SEQ ID NO: 532 - RNA, 21 nt, synthetic construct
  source 1..21: mol_type = other RNA
tatgctgtctgagaagcagca

SEQ ID NO: 533 - RNA, 16 nt, synthetic construct
  source 1..16: mol_type = other RNA
gctgcttctcagacaa

SEQ ID NO: 534 - RNA, 21 nt, synthetic construct
  source 1..21: mol_type = other RNA
ttgtctgagaagcagcagggc

SEQ ID NO: 535 - RNA, 16 nt, synthetic construct
  source 1..16: mol_type = other RNA
aggagggaaacatgga

SEQ ID NO: 536 - RNA, 21 nt, synthetic construct
  source 1..21: mol_type = other RNA
tccatgtttccctcctggttg

SEQ ID NO: 537 - RNA, 16 nt, synthetic construct
  source 1..16: mol_type = other RNA
caggagggaaacatga

SEQ ID NO: 538 - RNA, 21 nt, synthetic construct
  source 1..21: mol_type = other RNA
tcatgtttccctcctggttga

SEQ ID NO: 539 - RNA, 16 nt, synthetic construct
  source 1..16: mol_type = other RNA
ctgatttccctgacca

SEQ ID NO: 540 - RNA, 21 nt, synthetic construct
  source 1..21: mol_type = other RNA
tggtcagggaaatcaggacca

SEQ ID NO: 541 - RNA, 16 nt, synthetic construct
  source 1..16: mol_type = other RNA
cctggtcctgatttca

SEQ ID NO: 542 - RNA, 21 nt, synthetic construct
  source 1..21: mol_type = other RNA
tgaaatcaggaccaggcgagg

SEQ ID NO: 543 - RNA, 16 nt, synthetic construct
  source 1..16: mol_type = other RNA
agcctacacaaaggaa

SEQ ID NO: 544 - RNA, 21 nt, synthetic construct
  source 1..21: mol_type = other RNA
ttcctttgtgtaggctgcact

SEQ ID NO: 545 - RNA, 16 nt, synthetic construct
  source 1..16: mol_type = other RNA
cagcctacacaaagga

SEQ ID NO: 546 - RNA, 21 nt, synthetic construct
  source 1..21: mol_type = other RNA
tcctttgtgtaggctgcactg

SEQ ID NO: 547 - RNA, 16 nt, synthetic construct
  source 1..16: mol_type = other RNA
gtgcagcctacacaaa

SEQ ID NO: 548 - RNA, 21 nt, synthetic construct
  source 1..21: mol_type = other RNA
tttgtgtaggctgcactgaga

SEQ ID NO: 549 - RNA, 16 nt, synthetic construct
  source 1..16: mol_type = other RNA
agtgcagcctacacaa

SEQ ID NO: 550 - RNA, 21 nt, synthetic construct
  source 1..21: mol_type = other RNA
ttgtgtaggctgcactgagag

SEQ ID NO: 551 - RNA, 16 nt, synthetic construct
  source 1..16: mol_type = other RNA
ccctgactctcagtga

SEQ ID NO: 552 - RNA, 21 nt, synthetic construct
  source 1..21: mol_type = other RNA
tcactgagagtcagggtgtca

SEQ ID NO: 553 - RNA, 16 nt, synthetic construct
  source 1..16: mol_type = other RNA
accctgactctcagta

SEQ ID NO: 554 - RNA, 21 nt, synthetic construct
  source 1..21: mol_type = other RNA
tactgagagtcagggtgtcac

SEQ ID NO: 555 - RNA, 16 nt, synthetic construct
  source 1..16: mol_type = other RNA
aaacgcccaccacaaa

SEQ ID NO: 556 - RNA, 21 nt, synthetic construct
  source 1..21: mol_type = other RNA
tttgtggtgggcgttttgata

SEQ ID NO: 557 - RNA, 16 nt, synthetic construct
  source 1..16: mol_type = other RNA
gcacaagtgcagagta

SEQ ID NO: 558 - RNA, 21 nt, synthetic construct
  source 1..21: mol_type = other RNA
tactctgcacttgtgcactgc

SEQ ID NO: 559 - RNA, 16 nt, synthetic construct
  source 1..16: mol_type = other RNA
ggtgcacttcgagcca

SEQ ID NO: 560 - RNA, 21 nt, synthetic construct
  source 1..21: mol_type = other RNA
tggctcgaagtgcaccaggcg

SEQ ID NO: 561 - RNA, 16 nt, synthetic construct
  source 1..16: mol_type = other RNA
gcctggtgcacttcga

SEQ ID NO: 562 - RNA, 21 nt, synthetic construct
  source 1..21: mol_type = other RNA
tcgaagtgcaccaggcggtag

SEQ ID NO: 563 - RNA, 16 nt, synthetic construct
  source 1..16: mol_type = other RNA
cgcctggtgcacttca

SEQ ID NO: 564 - RNA, 21 nt, synthetic construct
  source 1..21: mol_type = other RNA
tgaagtgcaccaggcggtagg

SEQ ID NO: 565 - RNA, 16 nt, synthetic construct
  source 1..16: mol_type = other RNA
ccgcctggtgcactta

SEQ ID NO: 566 - RNA, 21 nt, synthetic construct
  source 1..21: mol_type = other RNA
taagtgcaccaggcggtaggg

SEQ ID NO: 567 - RNA, 16 nt, synthetic construct
  source 1..16: mol_type = other RNA
accgcctggtgcacta

SEQ ID NO: 568 - RNA, 21 nt, synthetic construct
  source 1..21: mol_type = other RNA
tagtgcaccaggcggtagggc

SEQ ID NO: 569 - RNA, 16 nt, synthetic construct
  source 1..16: mol_type = other RNA
cgacccaaggaccaga

SEQ ID NO: 570 - RNA, 21 nt, synthetic construct
  source 1..21: mol_type = other RNA
tctggtccttgggtcggaaca

SEQ ID NO: 571 - RNA, 16 nt, synthetic construct
  source 1..16: mol_type = other RNA
ccgacccaaggaccaa

SEQ ID NO: 572 - RNA, 21 nt, synthetic construct
  source 1..21: mol_type = other RNA
ttggtccttgggtcggaacaa

SEQ ID NO: 573 - RNA, 16 nt, synthetic construct
  source 1..16: mol_type = other RNA
tggcggatctcaacta

SEQ ID NO: 574 - RNA, 21 nt, synthetic construct
  source 1..21: mol_type = other RNA
tagttgagatccgccagcgac

SEQ ID NO: 575 - RNA, 16 nt, synthetic construct
  source 1..16: mol_type = other RNA
gtgacgtggaactgaa

SEQ ID NO: 576 - RNA, 21 nt, synthetic construct
  source 1..21: mol_type = other RNA
ttcagttccacgtcaccaata

SEQ ID NO: 577 - RNA, 16 nt, synthetic construct
  source 1..16: mol_type = other RNA
ttggtgacgtggaaca

SEQ ID NO: 578 - RNA, 21 nt, synthetic construct
  source 1..21: mol_type = other RNA
tgttccacgtcaccaataaga

SEQ ID NO: 579 - RNA, 16 nt, synthetic construct
  source 1..16: mol_type = other RNA
ccagatgcattttaaa

SEQ ID NO: 580 - RNA, 21 nt, synthetic construct
  source 1..21: mol_type = other RNA
tttaaaatgcatctggaacaa

SEQ ID NO: 581 - RNA, 16 nt, synthetic construct
  source 1..16: mol_type = other RNA
ggccagtaatgggaaa

SEQ ID NO: 582 - RNA, 21 nt, synthetic construct
  source 1..21: mol_type = other RNA
tttcccattactggcccagca

SEQ ID NO: 583 - RNA, 16 nt, synthetic construct
  source 1..16: mol_type = other RNA
gggccagtaatgggaa

SEQ ID NO: 584 - RNA, 21 nt, synthetic construct
  source 1..21: mol_type = other RNA
ttcccattactggcccagcag

SEQ ID NO: 585 - RNA, 16 nt, synthetic construct
  source 1..16: mol_type = other RNA
accatcaaagtgggaa

SEQ ID NO: 586 - RNA, 21 nt, synthetic construct
  source 1..21: mol_type = other RNA
ttcccactttgatggtccctg

SEQ ID NO: 587 - RNA, 16 nt, synthetic construct
  source 1..16: mol_type = other RNA
gaccatcaaagtggga

SEQ ID NO: 588 - RNA, 21 nt, synthetic construct
  source 1..21: mol_type = other RNA
tcccactttgatggtccctgg

SEQ ID NO: 589 - RNA, 16 nt, synthetic construct
  source 1..16: mol_type = other RNA
tggaaaacccagggaa

SEQ ID NO: 590 - RNA, 21 nt, synthetic construct
  source 1..21: mol_type = other RNA
ttccctgggttttccagcaca

SEQ ID NO: 591 - RNA, 16 nt, synthetic construct
  source 1..16: mol_type = other RNA
ctggaaaacccaggga

SEQ ID NO: 592 - RNA, 21 nt, synthetic construct
  source 1..21: mol_type = other RNA
tccctgggttttccagcacaa

SEQ ID NO: 593 - RNA, 16 nt, synthetic construct
  source 1..16: mol_type = other RNA
cgctggaaacactgaa

SEQ ID NO: 594 - RNA, 21 nt, synthetic construct
  source 1..21: mol_type = other RNA
ttcagtgtttccagcggttcc

SEQ ID NO: 595 - RNA, 16 nt, synthetic construct
  source 1..16: mol_type = other RNA
ccgctggaaacactga

SEQ ID NO: 596 - RNA, 21 nt, synthetic construct
  source 1..21: mol_type = other RNA
tcagtgtttccagcggttcct

SEQ ID NO: 597 - RNA, 16 nt, synthetic construct
  source 1..16: mol_type = other RNA
accgctggaaacacta

SEQ ID NO: 598 - RNA, 21 nt, synthetic construct
  source 1..21: mol_type = other RNA
tagtgtttccagcggttcctt

SEQ ID NO: 599 - RNA, 16 nt, synthetic construct
  source 1..16: mol_type = other RNA
aaccgctggaaacaca

SEQ ID NO: 600 - RNA, 21 nt, synthetic construct
  source 1..21: mol_type = other RNA
tgtgtttccagcggttccttc